European Patent Application EP 4 588 520 A2, published July 23, 2025. Title: Composition modulating botulinum neurotoxin effect. Applicant: FASTOX PHARMA SA. The sequence listing filed with the application follows.

SEQUENCE LISTING (95 sequences)

SEQ ID NO: 1 - protein, 21 aa, Azemiopsin
DNWWPKPPHQGPRPPRPRPKP

SEQ ID NO: 2 - protein, 22 aa, synthetic construct
  REGION 1..22: note = Consensus sequence for Wagglerin-1
  SITE 10: note = misc_feature - Xaa can be any naturally occurring amino acid
GGKPDLRPCXPPCHYIPRPKPR

SEQ ID NO: 3 - protein, 22 aa, Wagglerin-1
GGKPDLRPCHPPCHYIPRPKPR

SEQ ID NO: 4 - protein, 74 aa, alpha-bungarotoxin
IVCHTTATSPISAVTCPPGENLCYRKMWCDAFCSSRGKVVELGCAATCPSKKPYEEVTCCSTDKCNPHPKQRPG

SEQ ID NO: 5 - protein, 32 aa, alphaC-Conotoxin PrXA
TYGIYDAKPPFSCAGLRGGCVLPPNLRPKFKE

SEQ ID NO: 6 - protein, 71 aa, alpha-cobratoxin
IRCFITPDITSKDCPNGHVCYTKTWCDAFCSIRGKRVDLGCAATCPTVKTGVDIQCCSTDNCNPFPTRKRP

SEQ ID NO: 7 - protein, 19 aa, synthetic construct
  REGION 1..19: note = Consensus sequence for alpha-conotoxin GI or alpha-conotoxin MI
  SITE 1: note = MISC_FEATURE - X=absent or G
  SITE 2: note = MISC_FEATURE - X=absent or D or N or S or R
  SITE 3: note = MISC_FEATURE - X=absent or G
  SITE 4: note = MISC_FEATURE - X=absent or E or R or Y or I
  SITE 7: note = MISC_FEATURE - X=N or H
  SITE 11: note = MISC_FEATURE - X=G or A
  SITE 12: note = MISC_FEATURE - X=absent or G or A
  SITE 13: note = MISC_FEATURE - X=R or K or P
  SITE 14: note = MISC_FEATURE - X=H or Y or N or K
  SITE 15: note = MISC_FEATURE - X=Y or F
  SITE 16: note = MISC_FEATURE - X=S or N or K or D
  SITE 18: note = MISC_FEATURE - X=absent or G
  SITE 19: note = MISC_FEATURE - X=absent or K or R
XXXXCCXPACXXXXXXCXX

SEQ ID NO: 8 - protein, 14 aa, alpha-Conotoxin MI
GRCCHPACGKNYSC

SEQ ID NO: 9 - protein, 13 aa, alpha-Conotoxin GI
ECCNPACGRHYSC

SEQ ID NO: 10 - protein, 22 aa, Psi-conotoxin-PrIIIE
AARCCTYHGSCLKEKCRRKYCC

SEQ ID NO: 11 - protein, 67 aa, synthetic construct
  REGION 1..67: note = Consensus sequence for Candoxin
  SITE 1: note = MISC_FEATURE - X=M or I
  SITE 7: note = MISC_FEATURE - X=N or H or Q
  SITE 9: note = MISC_FEATURE - X=D or N
  SITE 13: note = MISC_FEATURE - X=A or P
  SITE 20: note = MISC_FEATURE - X=A or S
  SITE 21: note = MISC_FEATURE - X=S or G
  SITE 22: note = MISC_FEATURE - X=G or E
  SITE 24: note = MISC_FEATURE - X=K or I
  SITE 32: note = MISC_FEATURE - X=R or S
  SITE 33: note = MISC_FEATURE - X=E or T
  SITE 44: note = MISC_FEATURE - X=A or T
  SITE 55: note = MISC_FEATURE - X=L or N
  SITE 62: note = MISC_FEATURE - X=T or I
  SITE 64: note = MISC_FEATURE - X=D or E
  SITE 67: note = MISC_FEATURE - X=absent or I
XKCKICXFXTCRXGELKVCXXXEXYCFKESWXXARGTRIERGCXATCPKGSVYGXYVLCCTXDXCNX

SEQ ID NO: 12 - protein, 66 aa, Candoxin
MKCKICNFDTCRAGELKVCASGEKYCFKESWREARGTRIERGCAATCPKGSVYGLYVLCCTTDDCN

SEQ ID NO: 13 - protein, 65 aa, synthetic construct
  REGION 1..65: note = Consensus sequence for Haditoxin
  SITE 1: note = MISC_FEATURE - X=T or K
  SITE 2: note = MISC_FEATURE - X=K or I or L or T
  SITE 4: note = MISC_FEATURE - X=Y or F
  SITE 6: note = MISC_FEATURE - X=H or D
  SITE 7: note = MISC_FEATURE - X=Q or L or D
  SITE 8: note = MISC_FEATURE - X=S or T or L
  SITE 9: note = MISC_FEATURE - X=T or R
  SITE 10: note = MISC_FEATURE - X=T or N
  SITE 11: note = MISC_FEATURE - X=P or S
  SITE 12: note = MISC_FEATURE - X=E or K
  SITE 16: note = MISC_FEATURE - X=I or L
  SITE 18: note = MISC_FEATURE - X=P or G or R
  SITE 19: note = MISC_FEATURE - X=D or H
  SITE 21: note = MISC_FEATURE - X=G or W or M or V
  SITE 25: note = MISC_FEATURE - X=Y or F
  SITE 27: note = MISC_FEATURE - X=S or I or N
  SITE 29: note = MISC_FEATURE - X=W or L
  SITE 30: note = MISC_FEATURE - X=I or A
  SITE 31: note = MISC_FEATURE - X=D or Y or A
  SITE 32: note = MISC_FEATURE - X=G or R
  SITE 33: note = MISC_FEATURE - X=R or N or G
  SITE 34: note = MISC_FEATURE - X=E or D or V
  SITE 35: note = MISC_FEATURE - X=G or V or E
  SITE 36: note = MISC_FEATURE - X=R or K
  SITE 38: note = MISC_FEATURE - X=E or K
  SITE 42: note = MISC_FEATURE - X=T or S
  SITE 43: note = MISC_FEATURE - X=F or L
  SITE 47: note = MISC_FEATURE - X=E or D
  SITE 48: note = MISC_FEATURE - X=L or I
  SITE 49: note = MISC_FEATURE - X=T or R or K
  SITE 50: note = MISC_FEATURE - X=P or S or Y
  SITE 51: note = MISC_FEATURE - X=N or T
  SITE 53: note = MISC_FEATURE - X=K or I
  SITE 55: note = MISC_FEATURE - X=V or I
  SITE 59: note = MISC_FEATURE - X=R or T
  SITE 62: note = MISC_FEATURE - X=K or N
  SITE 65: note = MISC_FEATURE - X=Q or D or A
XXCXNXXXXXXXTTEXCXXSXYFCXKXSXXXXXXXXIXRGCXXTCPXXXXXGXYXYCCXRDXCNX

SEQ ID NO: 14 - protein, 65 aa, Haditoxin
TKCYNHQSTTPETTEICPDSGYFCYKSSWIDGREGRIERGCTFTCPELTPNGKYVYCCRRDKCNQ

SEQ ID NO: 15 - protein, 33 aa, synthetic construct
  REGION 1..33: note = Consensus sequence for Imperacalcin
  SITE 1: note = MISC_FEATURE - X=G or A or K or R
  SITE 2: note = MISC_FEATURE - X=D or N or S
  SITE 4: note = MISC_FEATURE - X=L or I or K
  SITE 5: note = MISC_FEATURE - X=P or A or K or E
  SITE 6: note = MISC_FEATURE - X=H or N or K
  SITE 7: note = MISC_FEATURE - X=L or R
  SITE 8: note = MISC_FEATURE - X=K or Q or R
  SITE 9: note = MISC_FEATURE - X=R or L or I
  SITE 11: note = MISC_FEATURE - X=K or R
  SITE 12: note = MISC_FEATURE - X=A or E or K or N or T
  SITE 13: note = MISC_FEATURE - X=D or N or T
  SITE 14: note = MISC_FEATURE - X=N or K or R
  SITE 15: note = MISC_FEATURE - X=D or E or Q
  SITE 18: note = MISC_FEATURE - X=G or S
  SITE 19: note = MISC_FEATURE - X=K or N
  SITE 20: note = MISC_FEATURE - X=K or S or N
  SITE 22: note = MISC_FEATURE - X=K or S or V
  SITE 26: note = MISC_FEATURE - X=T or A or R
  SITE 27: note = MISC_FEATURE - X=N or Q or I
  SITE 28: note = MISC_FEATURE - X=A or P or I
  SITE 29: note = MISC_FEATURE - X=E or S
  SITE 30: note = MISC_FEATURE - X=K or Q
  SITE 31: note = MISC_FEATURE - X=R or K
  SITE 33: note = MISC_FEATURE - X=R or E
XXCXXXXXXCXXXXXCCXXXCXRRGXXXXXXCX

SEQ ID NO: 16 - protein, 33 aa, Imperacalcin
GDCLPHLKRCKADNDCCGKKCKRRGTNAEKRCR

SEQ ID NO: 17 - protein, 104 aa, synthetic construct
  REGION 1..104: note = Consensus for Phospholipase A2 (large subunit) or Phospholipase A2 imperatoxin-1 or Heteromtoxin (large subunit)
  SITE 1: note = MISC_FEATURE - X=T or I
  SITE 2: note = MISC_FEATURE - X=M or V or I
  SITE 3: note = MISC_FEATURE - X=W or L
  SITE 10: note = MISC_FEATURE - X=S or A
  SITE 12: note = MISC_FEATURE - X=N or S
  SITE 13: note = MISC_FEATURE - X=E or K
  SITE 15: note = MISC_FEATURE - X=I or T or A or E
  SITE 16: note = MISC_FEATURE - X=N or D or S
  SITE 17: note = MISC_FEATURE - X=Y or I or G or E
  SITE 18: note = MISC_FEATURE - X=T or S or I or G
  SITE 19: note = MISC_FEATURE - X=D or E
  SITE 22: note = MISC_FEATURE - X=Y or W or L
  SITE 23: note = MISC_FEATURE - X=F or W
  SITE 24: note = MISC_FEATURE - X=S or K or Y or N or D
  SITE 25: note = MISC_FEATURE - X=N or K
  SITE 26: note = MISC_FEATURE - X=L or V
  SITE 28: note = MISC_FEATURE - X=S or R or L or I
  SITE 32: note = MISC_FEATURE - X=T or E or D
  SITE 38: note = MISC_FEATURE - X=S or N
  SITE 40: note = MISC_FEATURE - X=P or A or G
  SITE 41: note = MISC_FEATURE - X=A or S
  SITE 43: note = MISC_FEATURE - X=E or Q or K
  SITE 44: note = MISC_FEATURE - X=T or S
  SITE 47: note = MISC_FEATURE - X=G or N
  SITE 49: note = MISC_FEATURE - X=T or K
  SITE 51: note = MISC_FEATURE - X=E or T
  SITE 53: note = MISC_FEATURE - X=K or I or T or A or V
  SITE 54: note = MISC_FEATURE - X=Y or F
  SITE 60: note = MISC_FEATURE - X=K or E or D
  SITE 63: note = MISC_FEATURE - X=S or A or T or D or E or K or V
  SITE 64: note = MISC_FEATURE - X=A or T or V or K
  SITE 66: note = MISC_FEATURE - X=E or Q or K or D or G
  SITE 67: note = MISC_FEATURE - X=K or Q or N
  SITE 70: note = MISC_FEATURE - X=R or K or S or D
  SITE 71: note = MISC_FEATURE - X=D or N or S
  SITE 72: note = MISC_FEATURE - X=V or I
  SITE 73: note = MISC_FEATURE - X=R or H or T or P or S or D
  SITE 75: note = MISC_FEATURE - X=I or P or G or V or T or Y or F
  SITE 76: note = MISC_FEATURE - X=L or M or F or I or W
  SITE 77: note = MISC_FEATURE - X=E or A or T or S
  SITE 78: note = MISC_FEATURE - X=G or Q or R or S or K
  SITE 79: note = MISC_FEATURE - X=K or P
  SITE 80: note = MISC_FEATURE - X=A or P
  SITE 81: note = MISC_FEATURE - X=A or V or I
  SITE 82: note = MISC_FEATURE - X=A or F or G or S
  SITE 83: note = MISC_FEATURE - X=A or T or F or M
  SITE 84: note = MISC_FEATURE - X=V or I
  SITE 85: note = MISC_FEATURE - X=R or K
  SITE 86: note = MISC_FEATURE - X=K or Y or F or M
  SITE 87: note = MISC_FEATURE - X=T or L or I or V
  SITE 90: note = MISC_FEATURE - X=D or G or E or T or N
  SITE 97: note = MISC_FEATURE - X=F or Y
  SITE 98: note = MISC_FEATURE - X=N or S
  SITE 99: note = MISC_FEATURE - X=V or L
  SITE 100: note = MISC_FEATURE - X=K or Q
  SITE 102: note = MISC_FEATURE - X=P or S or E
  SITE 103: note = MISC_FEATURE - X=S or A or N or G
  SITE 104: note = MISC_FEATURE - X=G or Q or E or A
XXXGTKWCGXGXXAXXXXXLGXXXXXDXCCRXHDHCDXIXXGXXKYXLXNXGXXTMMNCXCEXXFXXCLXXXXGXXXXXXXXXXXXXYFXLYGNGCXXXXCXXX

SEQ ID NO: 18 - protein, 104 aa, Phospholipase A2 imperatoxin-1 large subunit
TMWGTKWCGSGNEATDISELGYWSNLDSCCRTHDHCDNIPSGQTKYGLTNEGKYTMMNCKCETAFEQCLRNVTGGMEGPAAGFVRKTYFDLYGNGCYNVQCPSQ

SEQ ID NO: 19 - protein, 104 aa, Heteromtoxin large subunit
TVWGTKWCGSGNEATSGIDLGYFKNLDSCCRTHDHCDNIPAGETKYGLTNEGIYTMMNCKCESVFKQCLKDVTGVFEGPAAAAVRKIYFDLYGNGCYSVQCPAG

SEQ ID NO: 20 - protein, 103 aa, Phospholipase A2 large subunit
TMWGTKWCGSGNKAINYTDLGYFSNLDSCCRTHDHCDNIAAGETKYGLTNEGKYTMMNCKCEATFQQCLRDVHGPLEGKAAFTIRKLYFGLYGNGCFNVQCPS

SEQ ID NO: 21 - protein, 104 aa, Phospholipase A2
TMWGTKWCGSGNEAINYTDLGYFSNLDSCCRTHDHCDSIPAGETKYGLTNEGKYTMMNCKCESAFEKCLRDVRGILEGKAAAAVRKTYFDLYGNGCFNVKCPSG

SEQ ID NO: 22 - protein, 36 aa, synthetic construct
  REGION 1..36: note = Consensus sequnce for Insecticidal Toxin LaIT1 or Phi-Liotoxin-Lw1a
  SITE 10: note = MISC_FEATURE - X=T or S
  SITE 18: note = MISC_FEATURE - X=Q or K
  SITE 33: note = MISC_FEATURE - X=K or N
DFPLSKEYEXCVRPRKCXPPLKCNKAQICVDPXKGW

SEQ ID NO: 23 - protein, 36 aa, Insecticidal Toxin LaIT1
DFPLSKEYETCVRPRKCQPPLKCNKAQICVDPKKGW

SEQ ID NO: 24 - protein, 36 aa, Phi-Liotoxin-Lw1a
DFPLSKEYESCVRPRKCKPPLKCNKAQICVDPNKGW

SEQ ID NO: 25 - protein, 60 aa, synthetic construct
  REGION 1..60: note = Consensus sequence for Calciseptine or Toxin FS2
  SITE 5: note = MISC_FEATURE - X=I or Sor T
  SITE 8: note = MISC_FEATURE - X=A or S
  SITE 9: note = MISC_FEATURE - X=S or L
  SITE 10: note = MISC_FEATURE - X=L or Q
  SITE 11: note = MISC_FEATURE - X=P or A
  SITE 12: note = MISC_FEATURE - X=R or K
  SITE 13: note = MISC_FEATURE - X=A or T
  SITE 16: note = MISC_FEATURE - X=T or S
  SITE 18: note = MISC_FEATURE - X=V or E
  SITE 19: note = MISC_FEATURE - X=E or G
  SITE 21: note = MISC_FEATURE - X=T or S
  SITE 30: note = MISC_FEATURE - X=Q or H or S
  SITE 31: note = MISC_FEATURE - X=R or P
  SITE 32: note = MISC_FEATURE - X=E or Q or D
  SITE 36: note = MISC_FEATURE - X=E or D
  SITE 51: note = MISC_FEATURE - X=E or A
RICYXHKXXXXXXTKXCXXNXCYKMFIRTXXXYISXRGCGCPTAMWPYQTXCCKGDRCNK

SEQ ID NO: 26 - protein, 60 aa, Calsiseptine
RICYIHKASLPRATKTCVENTCYKMFIRTQREYISERGCGCPTAMWPYQTECCKGDRCNK

SEQ ID NO: 27 - protein, 60 aa, Toxin FS2
RICYSHKASLPRATKTCVENTCYKMFIRTHRQYISERGCGCPTAMWPYQTECCKGDRCNK

SEQ ID NO: 28 - protein, 56 aa, synthetic construct
  REGION 1..56: note = Consensus sequence for Vasotab
  SITE 2: note = MISC_FEATURE - X=E or D or N
  SITE 5: note = MISC_FEATURE - X=R or T
  SITE 6: note = MISC_FEATURE - X=I or V
  SITE 9: note = MISC_FEATURE - X=A or S
  SITE 11: note = MISC_FEATURE - X=Y or F
  SITE 12: note = MISC_FEATURE - X=R or T
  SITE 30: note = MISC_FEATURE - X=G or A
  SITE 34: note = MISC_FEATURE - X=S or G
  SITE 36: note = MISC_FEATURE - X=N or D
  SITE 37: note = MISC_FEATURE - X=A or S
  SITE 45: note = MISC_FEATURE - X=D or A
DXCPXXCTXDXXPVCGTPSGGRRSANRTFXNQCXLXXHNCLNKGXTYDKLHDGECK

SEQ ID NO: 29 - protein, 56 aa, Vasotab
DECPRICTADYRPVCGTPSGGRRSANRTFGNQCSLNAHNCLNKGDTYDKLHDGECK

SEQ ID NO: 30 - protein, 12 aa, synthetic construct
  REGION 1..12: note = Consensus sequence for Glacontryphan M
  SITE 1: note = MISC_FEATURE - X=N or R or I or H
  SITE 2: note = MISC_FEATURE - X=E or R
  SITE 3: note = MISC_FEATURE - X=S or N
  SITE 4: note = MISC_FEATURE - X=E or G
  SITE 8: note = MISC_FEATURE - X=H or R or K or Q
XXXXCPWXPWCG

SEQ ID NO: 31 - protein, 12 aa, Glacontryphan M
NESECPWHPWCG

SEQ ID NO: 32 - protein, 26 aa, omega-conotoxin-TxVII
CKQADEPCDVFSLDCCTGICLGVCMW

SEQ ID NO: 33 - protein, 65 aa, synthetic construct
  REGION 1..65: note = Consensus sequence for Omega-ctenitoxin-Cs1a
  SITE 1: note = MISC_FEATURE - X=S or D
  SITE 7: note = MISC_FEATURE - X=E or H
  SITE 11: note = MISC_FEATURE - X=N or S
  SITE 12: note = MISC_FEATURE - X=D or N
  SITE 15: note = MISC_FEATURE - X=N or G
  SITE 19: note = MISC_FEATURE - X=K or G
  SITE 20: note = MISC_FEATURE - X=G or H
  SITE 24: note = MISC_FEATURE - X=L or Y
  SITE 29: note = MISC_FEATURE - X=S or T
  SITE 31: note = MISC_FEATURE - X=F or V
  SITE 32: note = MISC_FEATURE - X=D or V
  SITE 33: note = MISC_FEATURE - X=D or T
  SITE 34: note = MISC_FEATURE - X=E or Q or H
  SITE 37: note = MISC_FEATURE - X=Q or E
  SITE 38: note = MISC_FEATURE - X=P or E or G
  SITE 43: note = MISC_FEATURE - X=A or F
  SITE 46: note = MISC_FEATURE - X=R or T
  SITE 48: note = MISC_FEATURE - X=M or P
  SITE 49: note = MISC_FEATURE - X=G or H or R
  SITE 51: note = MISC_FEATURE - X=Q or K
  SITE 53: note = MISC_FEATURE - X=I or A
  SITE 55: note = MISC_FEATURE - X=T or L
  SITE 56: note = MISC_FEATURE - X=G or V
  SITE 57: note = MISC_FEATURE - X=L or V
  SITE 58: note = MISC_FEATURE - X=N or G
  SITE 59: note = MISC_FEATURE - X=I or F
  SITE 60: note = MISC_FEATURE - X=F or G
  SITE 61: note = MISC_FEATURE - X=R or K
  SITE 62: note = MISC_FEATURE - X=G or K
  SITE 63: note = MISC_FEATURE - X=L or I
  SITE 65: note = MISC_FEATURE - X=K or G
XCIPKHXECTXXKHXCCRXXLFKXKCQCXTXXXXSGXXTERCXCGXPXXHXAXEXXXXXXXXXFX

SEQ ID NO: 34 - protein, 65 aa, omega-ctenitoxin-Cs1a
SCIPKHEECTNDKHNCCRKGLFKLKCQCSTFDDESGQPTERCACGRPMGHQAIETGLNIFRGLFK

SEQ ID NO: 35 - protein, 19 aa, U7-ctenitoxin-Pn1b
GCIGRNESQKKDNVYKFKE

SEQ ID NO: 36 - protein, 40 aa, synthetic construct
  REGION 1..40: note = Consensus sequence for Kappa-ctenitoxin-Pn1a or U9-ctenitoxin-Pn1a or U6-ctenitoxin-Pn1a
  SITE 1: note = MISC_FEATURE - X=E or A or G or S or K or N
  SITE 3: note = MISC_FEATURE - X=absent or I
  SITE 5: note = MISC_FEATURE - X=A or G or D or K or E
  SITE 6: note = MISC_FEATURE - X=V or L or A or D
  SITE 7: note = MISC_FEATURE - X=Y or W
  SITE 8: note = MISC_FEATURE - X=E or K or G
  SITE 9: note = MISC_FEATURE - X=R or K or S or E
  SITE 11: note = MISC_FEATURE - X=G or N or D or K or T or W
  SITE 12: note = MISC_FEATURE - X=K or H or S or N or W or Y
  SITE 13: note = MISC_FEATURE - X=absent or G or P
  SITE 14: note = MISC_FEATURE - X=absent or Y or A or V or G or E
  SITE 15: note = MISC_FEATURE - X=K or S or N or R or L or T
  SITE 16: note = MISC_FEATURE - X=R or P or T or K
  SITE 19: note = MISC_FEATURE - X=E or D or N or V or R or K
  SITE 20: note = MISC_FEATURE - X=absent or G
  SITE 21: note = MISC_FEATURE - X=absent or Y or V
  SITE 22: note = MISC_FEATURE - X=absent or N
  SITE 23: note = MISC_FEATURE - X=absent or G
  SITE 24: note = MISC_FEATURE - X=absent or Y
  SITE 25: note = MISC_FEATURE - X=E or D or N or K or S or G
  SITE 27: note = MISC_FEATURE - X=P or A or T or G
  SITE 29: note = MISC_FEATURE - X=K or I or M or R or Q
  SITE 31: note = MISC_FEATURE - X=N or D or S or T
  SITE 32: note = MISC_FEATURE - X=absent or I or L or M
  SITE 33: note = MISC_FEATURE - X=absent or V or A or I or M or G
  SITE 34: note = MISC_FEATURE - X=M or G or A
  SITE 35: note = MISC_FEATURE - X=absent or D or G or S or T or N
  SITE 36: note = MISC_FEATURE - X=N or R or T
  SITE 38: note = MISC_FEATURE - X=T or I or K or N or E
  SITE 40: note = MISC_FEATURE - X=K or R or E or T
XCXAXXXXXCXXXXXXCCXXXXXXXRXCXCXXXXXXCXCX

SEQ ID NO: 37 - protein, 36 aa, U9-ctenitoxin-Pn1a
GCADAYKSCNHPRTCCDGYNGYKRACICSGSNCKCK

SEQ ID NO: 38 - protein, 34 aa, U6-ctenitoxin-Pn1a
ACADVYKECWYPEKPCCKDRACQCTLGMTCKCKA

SEQ ID NO: 39 - protein, 40 aa, Kappa-ctenitoxin-Pn1a
AECAAVYERCGKGYKRCCEERPCKCNIVMDNCTCKKFISE

SEQ ID NO: 40 - protein, 58 aa, synthetic construct
  REGION 1..58: note = Consensus sequence for Omega-ctenitoxin-Pr2a
  SITE 1: note = MISC_FEATURE - X=A or G
  SITE 3: note = MISC_FEATURE - X=I or L
  SITE 4: note = MISC_FEATURE - X=P or A or D
  SITE 5: note = MISC_FEATURE - X=R or I
  SITE 7: note = MISC_FEATURE - X=E or K
  SITE 8: note = MISC_FEATURE - X=I or T
  SITE 10: note = MISC_FEATURE - X=T or K
  SITE 17: note = MISC_FEATURE - X=G or D
  SITE 19: note = MISC_FEATURE - X=D or G
  SITE 21: note = MISC_FEATURE - X=Q or V
  SITE 26: note = MISC_FEATURE - X=P or F
  SITE 27: note = MISC_FEATURE - X=G or D
  SITE 28: note = MISC_FEATURE - X=S or W
  SITE 29: note = MISC_FEATURE - X=absent or F
  SITE 30: note = MISC_FEATURE - X=absent or G
  SITE 31: note = MISC_FEATURE - X=absent or G
  SITE 32: note = MISC_FEATURE - X=S or K
  SITE 33: note = MISC_FEATURE - X=L or W
  SITE 34: note = MISC_FEATURE - X=G or H or Q
  SITE 35: note = MISC_FEATURE - X=I or P
  SITE 36: note = MISC_FEATURE - X=F or V
  SITE 37: note = MISC_FEATURE - X=K or G
  SITE 42: note = MISC_FEATURE - X=H or Y
  SITE 43: note = MISC_FEATURE - X=A or T or G
  SITE 44: note = MISC_FEATURE - X=N or L
  SITE 45: note = MISC_FEATURE - X=K or Q
  SITE 47: note = MISC_FEATURE - X=F or V
  SITE 49: note = MISC_FEATURE - X=N or D or A
  SITE 50: note = MISC_FEATURE - X=R or H
  SITE 52: note = MISC_FEATURE - X=K or Q
  SITE 53: note = MISC_FEATURE - X=E or K
  SITE 56: note = MISC_FEATURE - X=K or P
  SITE 57: note = MISC_FEATURE - X=K or N
  SITE 58: note = MISC_FEATURE - X=A or V
XCXXXGXXCXDDCECCXCXNXCYCPXXXXXXXXXXXXCSCAXXXXYXCXXKXXKCXXX

SEQ ID NO: 41 - protein, 55 aa, omega-ctenitoxin-Pr2a
ACIPRGEICTDDCECCGCDNECYCPIGSSLGIFKCSCAHANKYFCNRKKEKCKKA

SEQ ID NO: 42 - protein, 60 aa, synthetic construct; identical to SEQ ID NO: 25
  REGION 1..60: note = Consensus sequence for Toxin C10S2C2 or Toxin S4C8
  SITE 5: note = MISC_FEATURE - X=I or S or T
  SITE 8: note = MISC_FEATURE - X=A or S
  SITE 9: note = MISC_FEATURE - X=S or L
  SITE 10: note = MISC_FEATURE - X=L or Q
  SITE 11: note = MISC_FEATURE - X=P or A
  SITE 12: note = MISC_FEATURE - X=R or K
  SITE 13: note = MISC_FEATURE - X=A or T
  SITE 16: note = MISC_FEATURE - X=T or S
  SITE 18: note = MISC_FEATURE - X=V or E
  SITE 19: note = MISC_FEATURE - X=E or G
  SITE 21: note = MISC_FEATURE - X=T or S
  SITE 30: note = MISC_FEATURE - X=Q or H or S
  SITE 31: note = MISC_FEATURE - X=R or P
  SITE 32: note = MISC_FEATURE - X=E or Q or D
  SITE 36: note = MISC_FEATURE - X=E or D
  SITE 51: note = MISC_FEATURE - X=E or A

SEQ ID NO: 43 - protein, 60 aa, Toxin S4C8
RICYTHKSLQAKTTKSCEGNTCYKMFIRTSREYISERGCGCPTAMWPYQTECCKGDRCNK

SEQ ID NO: 44 - protein, 60 aa, Toxin C10S2C2
RICYSHKASLPRATKTCVENSCYKMFIRTSPDYISDRGCGCPTAMWPYQTACCKGDRCNK

SEQ ID NO: 45 - protein, 23 aa, synthetic construct
  REGION 1..23: note = Consensus sequence for mu-conotoxin GIIIb or mu-conotoxin TIIIA or mu-conotoxin PIIIa
  SITE 1: note = MISC_FEATURE - X=absent or R or E or Q
  SITE 2: note = MISC_FEATURE - X=R or H
  SITE 3: note = MISC_FEATURE - X=D or G or V or L
  SITE 6: note = MISC_FEATURE - X=T or K or N or G
  SITE 7: note = MISC_FEATURE - X=P or G or Y or F
  SITE 9: note = MISC_FEATURE - X=K or R or E or Q or M
  SITE 10: note = MISC_FEATURE - X=K or G or S
  SITE 12: note = MISC_FEATURE - X=K or S or R
  SITE 13: note = MISC_FEATURE - X=D or S
  SITE 15: note = MISC_FEATURE - X=Q or R or E or H or A
  SITE 17: note = MISC_FEATURE - X=K or R
  SITE 18: note = MISC_FEATURE - X=P or N
  SITE 19: note = MISC_FEATURE - X=Q or M or L or K or S or H
  SITE 20: note = MISC_FEATURE - X=R or K or H or Q or Y
  SITE 23: note = MISC_FEATURE - X=absent or A
XXXCCXXPXXCXXRXCXXXXCCX

SEQ ID NO: 46 - protein, 22 aa, mu-conotoxin GIIIb
RDCCTPPRKCKDRRCKPMKCCA

SEQ ID NO: 47 - protein, 22 aa, mu-conotoxin PIIIa
QRLCCGFPKSCRSRQCKPHRCC

SEQ ID NO: 48 - protein, 22 aa, mu-conotoxin TIIIA
RHGCCKGPKGCSSRECRPQHCC

SEQ ID NO: 49 - protein, 35 aa, synthetic construct
  REGION 1..35: note = Consensus sequence for mu-Conotoxin GvIIJ
  SITE 1: note = MISC_FEATURE - X=G or D or W
  SITE 5: note = MISC_FEATURE - X=D or K
  SITE 6: note = MISC_FEATURE - X=P or A
  SITE 7: note = MISC_FEATURE - X=G or E
  SITE 8: note = MISC_FEATURE - X=A or D
  SITE 9: note = MISC_FEATURE - X=T or A
  SITE 12: note = MISC_FEATURE - X=K or T
  SITE 14: note = MISC_FEATURE - X=R or K or Y
  SITE 16: note = MISC_FEATURE - X=Y or R or K
  SITE 21: note = MISC_FEATURE - X=F or L or M
  SITE 23: note = MISC_FEATURE - X=D or N
  SITE 24: note = MISC_FEATURE - X=C or Q or K
  SITE 25: note = MISC_FEATURE - X=Y or A
  SITE 26: note = MISC_FEATURE - X=T or S or N
  SITE 27: note = MISC_FEATURE - X=K or G or W
  SITE 28: note = MISC_FEATURE - X=T or K
  SITE 30: note = MISC_FEATURE - X=K or T or L
  SITE 31: note = MISC_FEATURE - X=D or G or R
  SITE 32: note = MISC_FEATURE - X=absent or K
  SITE 33: note = MISC_FEATURE - X=absent or S
  SITE 34: note = MISC_FEATURE - X=absent or S
  SITE 35: note = MISC_FEATURE - X=absent or A
XWCGXXXXXCGXLXLXCCSGXCXXXXXXCXXXXXX

SEQ ID NO: 50 - protein, 35 aa, mu-conotoxin GvIIJ
GWCGDPGATCGKLRLYCCSGFCDCYTKTCKDKSSA

SEQ ID NO: 51 - protein, 32 aa, synthetic construct
  REGION 1..32: note = Consensus sequence for MuO-conotoxin MfVIA
  SITE 2: note = MISC_FEATURE - X=D or A
  SITE 4: note = MISC_FEATURE - X=Q or R or S
  SITE 5: note = MISC_FEATURE - X=E or K or A
  SITE 6: note = MISC_FEATURE - X=K or L
  SITE 8: note = MISC_FEATURE - X=E or D
  SITE 11: note = MISC_FEATURE - X=I or P
  SITE 14: note = MISC_FEATURE - X=I or F
  SITE 15: note = MISC_FEATURE - X=L or I
  SITE 16: note = MISC_FEATURE - X=G or S
  SITE 17: note = MISC_FEATURE - X=F or V or S
  SITE 18: note = MISC_FEATURE - X=V or I or G
  SITE 19: note = MISC_FEATURE - X=Y or D
  SITE 22: note = MISC_FEATURE - X=P or L or I
  SITE 28: note = MISC_FEATURE - X=P or H or L
  SITE 30: note = misc_feature - Xaa can be any naturally occurring amino acid
  SITE 32: note = misc_feature - Xaa can be any naturally occurring amino acid
RXCXXXWXYCXVPXXXXXXCCXGLICGXFXCX

SEQ ID NO: 52 - protein, 32 aa, muO-conotoxin MfVIA
RDCQEKWEYCIVPILGFVYCCPGLICGPFVCV

SEQ ID NO: 53 - protein, 31 aa, synthetic construct
  REGION 1..31: note = Consensus sequence for mu-conotoxin CnIIIc
  SITE 1: note = MISC_FEATURE - X=absent or V or I
  SITE 2: note = MISC_FEATURE - X=absent or T or G or V
  SITE 3: note = MISC_FEATURE - X=absent or D or E or Q or G or L or pyroglutamate (pGlu)
  SITE 4: note = MISC_FEATURE - X=absent or R or G or N or Y
  SITE 7: note = MISC_FEATURE - X=K or N or D or E or G or Q
  SITE 8: note = MISC_FEATURE - X=absent or K or P
  SITE 9: note = MISC_FEATURE - X=absent or K
  SITE 10: note = MISC_FEATURE - X=absent or G or P
  SITE 11: note = MISC_FEATURE - X=absent or N
  SITE 12: note = MISC_FEATURE - X=absent or G or V or E
  SITE 13: note = MISC_FEATURE - X=absent or K or P or R or Q
  SITE 14: note = MISC_FEATURE - X=absent or R or K or N or M
  SITE 15: note = MISC_FEATURE - X=absent or E or G or A or L or M
  SITE 17: note = MISC_FEATURE - X=absent or S or F
  SITE 18: note = MISC_FEATURE - X=G or S or T or N
  SITE 19: note = MISC_FEATURE - X=R or K
  SITE 22: note = MISC_FEATURE - X=R or K or E
  SITE 23: note = MISC_FEATURE - X=D or G or N or I
  SITE 24: note = MISC_FEATURE - X=H or N
  SITE 25: note = MISC_FEATURE - X=S or A
  SITE 26: note = MISC_FEATURE - X=R or Q
  SITE 29: note = MISC_FEATURE - X=absent or R
  SITE 30: note = MISC_FEATURE - X=absent or Q
  SITE 31: note = MISC_FEATURE - X=absent or Q
XXXXCCXXXXXXXXXCXXXWCXXXXXCCXXX

SEQ ID NO: 54 - protein, 22 aa, mu-conotoxin CnIIIc
ZGCCNGPKGCSSKWCRDHARCC

SEQ ID NO: 55 - protein, 41 aa, synthetic construct
  REGION 1..41: note = Consensus sequence for Mu-thomitoxin-Hme1a or Mu-thomitoxin-Hme1b or Mu-thomitoxin-Hme1c
  SITE 4: note = MISC_FEATURE - X=P or A
  SITE 5: note = MISC_FEATURE - X=Y or S or K
  SITE 6: note = MISC_FEATURE - X=G or F or N
  SITE 7: note = MISC_FEATURE - X=K or G
  SITE 8: note = MISC_FEATURE - X=T or E
  SITE 10: note = MISC_FEATURE - X=E or A
  SITE 11: note = MISC_FEATURE - X=F or W
  SITE 12: note = MISC_FEATURE - X=W or F
  SITE 15: note = MISC_FEATURE - X=P or E
  SITE 16: note = MISC_FEATURE - X=W or S
  SITE 19: note = MISC_FEATURE - X=A or T or G
  SITE 20: note = MISC_FEATURE - X=G or A
  SITE 21: note = MISC_FEATURE - X=K or I or L
  SITE 22: note = MISC_FEATURE - X=absent or S
  SITE 25: note = MISC_FEATURE - X=L or W or Y
  SITE 26: note = MISC_FEATURE - X=N or V or S
  SITE 27: note = MISC_FEATURE - X=V or F or I
  SITE 28: note = MISC_FEATURE - X=W or F or K
  SITE 29: note = MISC_FEATURE - X=S or T or R
  SITE 30: note = MISC_FEATURE - X=M or S or N
  SITE 31: note = MISC_FEATURE - X=T or K or L
  SITE 32: note = MISC_FEATURE - X=L or F or K
  SITE 33: note = MISC_FEATURE - X=S or M or I
  SITE 35: note = MISC_FEATURE - X=T or R or V
  SITE 36: note = MISC_FEATURE - X=absent or R
  SITE 37: note = MISC_FEATURE - X=absent or N or V
  SITE 38: note = MISC_FEATURE - X=absent or F or W
  SITE 39: note = MISC_FEATURE - X=absent or G
  SITE 40: note = MISC_FEATURE - X=absent or K
  SITE 41: note = MISC_FEATURE - X=absent or D
GCIXXXXXCXXXSGXXCCXXXXCKXXXXXXXXXCXXXXXXX

SEQ ID NO: 56 - protein, 37 aa, mu-thomitoxin-Hme1a
GCIPYGKTCEFWSGPWCCAGKCKLNVWSMTLSCTRNF

SEQ ID NO: 57 - protein, 40 aa, mu-thomitoxin-Hme1b
GCIPSFGECAWFSGESCCTGICKWVFFTSKFMCRRVWGKD

SEQ ID NO: 58 - protein, 35 aa, mu-thomitoxin-Hme1c
GCIAKNKECAWFSGEWCCGALSCKYSIKRNLKICV

SEQ ID NO: 59 - protein, 66 aa, synthetic construct
  REGION 1..66: note = Consensus sequence for Muscarinic toxin alpha or Muscarinic toxin 1 or Adrenergic toxin rho-elapitoxin-Dp1a or Toxin AdTx1 or Muscarinic toxin 2 or Muscarinic toxin 7 or Muscarinic toxin 3
  SITE 5: note = MISC_FEATURE - X=T or K
  SITE 6: note = MISC_FEATURE - X=S or K or E or T
  SITE 7: note = MISC_FEATURE - X=K or D or N
  SITE 8: note = MISC_FEATURE - X=S or T
  SITE 10: note = MISC_FEATURE - X=F or W or G
  SITE 11: note = MISC_FEATURE - X=G or F
  SITE 12: note = MISC_FEATURE - X=I or V or P
  SITE 14: note = MISC_FEATURE - X=T or S
  SITE 15: note = MISC_FEATURE - X=E or Q
  SITE 16: note = MISC_FEATURE - X=N or D
  SITE 19: note = MISC_FEATURE - X=D or A or P
  SITE 23: note = MISC_FEATURE - X=L or V
  SITE 26: note = MISC_FEATURE - X=K or I
  SITE 27: note = MISC_FEATURE - X=K or R
  SITE 28: note = MISC_FEATURE - X=W or R
  SITE 29: note = MISC_FEATURE - X=Y or H or Q
  SITE 30: note = MISC_FEATURE - X=Y or M
  SITE 31: note = MISC_FEATURE - X=L or I or V
  SITE 32: note = MISC_FEATURE - X=N or V or S or T or I
  SITE 33: note = MISC_FEATURE - X=H or P
  SITE 34: note = MISC_FEATURE - X=R or K or G
  SITE 35: note = MISC_FEATURE - X=Y or I or M or R or N
  SITE 36: note = MISC_FEATURE - X=S or T or Y
  SITE 37: note = MISC_FEATURE - X=D or E or K
  SITE 38: note = MISC_FEATURE - X=I or S or K or F
  SITE 39: note = MISC_FEATURE - X=T or I
  SITE 40: note = MISC_FEATURE - X=W or R or K
  SITE 43: note = MISC_FEATURE - X=A or T or V
  SITE 48: note = MISC_FEATURE - X=K or I
  SITE 49: note = MISC_FEATURE - X=P or A or V
  SITE 50: note = MISC_FEATURE - X=T or E or D
  SITE 51: note = MISC_FEATURE - X=N or Y
  SITE 52: note = MISC_FEATURE - X=absent or V
  SITE 53: note = MISC_FEATURE - X=R or Y or N
  SITE 54: note = MISC_FEATURE - X=E or D
  SITE 55: note = MISC_FEATURE - X=T or S or V or P
  SITE 57: note = MISC_FEATURE - X=H or R or E or N
  SITE 60: note = MISC_FEATURE - X=E or N or K or G or S
  SITE 62: note = MISC_FEATURE - X=D or E
  SITE 66: note = MISC_FEATURE - X=E or N or L or K or D
LTCVXXXXIXXXTXXXCPXGQNXCFXXXXXXXXXXXXXXXGCXATCPXXXXXXXXIXCCXTXKCNX

SEQ ID NO: 60 - protein, 66 aa, Muscarinic toxin alpha
LTCVTSKSIFGITTENCPDGQNLCFKKWYYLNHRYSDITWGCAATCPKPTNVRETIHCCETDKCNE

SEQ ID NO: 61 - protein, 39 aa, omega-theraphotoxin-Cc1a
GVDKEGCKYMFGSCGKSDDCCPKLACKRTFNYCAWDGSV

SEQ ID NO: 62 - protein, 66 aa, synthetic construct
  REGION 1..66: note = Consensus sequence for beta-mammal toxin Css2
  SITE 5: note = MISC_FEATURE - X=L or I
  SITE 7: note = MISC_FEATURE - X=S or D or N or E
  SITE 8: note = MISC_FEATURE - X=K or S or H or L or Y
  SITE 9: note = MISC_FEATURE - X=S or N or Y or H or G
  SITE 10: note = MISC_FEATURE - X=T or D
  SITE 14: note = MISC_FEATURE - X=Y or F
  SITE 15: note = MISC_FEATURE - X=E or A or T
  SITE 17: note = MISC_FEATURE - X=L or F or Y or A
  SITE 21: note = MISC_FEATURE - X=D or E
  SITE 26: note = MISC_FEATURE - X=L or K or V
  SITE 30: note = MISC_FEATURE - X=K or R
  SITE 31: note = MISC_FEATURE - X=Q or L or A
  SITE 32: note = MISC_FEATURE - X=Q or G or R
  SITE 33: note = MISC_FEATURE - X=Y or H
  SITE 34: note = MISC_FEATURE - X=G or Y
  SITE 35: note = MISC_FEATURE - X=K or Q
  SITE 36: note = MISC_FEATURE - X=absent or S or G
  SITE 37: note = MISC_FEATURE - X=S or A
  SITE 38: note = MISC_FEATURE - X=G or H
  SITE 45: note = MISC_FEATURE - X=A or G
  SITE 49: note = MISC_FEATURE - X=T or N
  SITE 50: note = MISC_FEATURE - X=H or Q
  SITE 56: note = MISC_FEATURE - X=V or I
  SITE 58: note = MISC_FEATURE - X=W or R
  SITE 61: note = MISC_FEATURE - X=P or K
  SITE 62: note = MISC_FEATURE - X=N or K
  SITE 64: note = MISC_FEATURE - X=T or R or K
  SITE 66: note = MISC_FEATURE - X=N or S or T or R or Y
KEGYXVXXXXGCKXXCXKLGXNDYCXRECXXXXXXXXXGYCYAFXCWCXXLYEQAXVXPLXXKXCX

SEQ ID NO: 63 - protein, 66 aa, beta-mammal toxin Css2
KEGYLVSKSTGCKYECLKLGDNDYCLRECKQQYGKSSGGYCYAFACWCTHLYEQAVVWPLPNKTCN

SEQ ID NO: 64 - protein, 66 aa, synthetic construct
  REGION 1..66: note = Consensus sequence for alpha-like toxin BmK-M1
  SITE 1: note = MISC_FEATURE - X=V or G or A
  SITE 2: note = MISC_FEATURE - X=R or S
  SITE 4: note = MISC_FEATURE - X=A or G
  SITE 8: note = MISC_FEATURE - X=K or Q or D or L
  SITE 9: note = MISC_FEATURE - X=P or N or D
  SITE 10: note = MISC_FEATURE - X=H or E or Y or K
  SITE 13: note = MISC_FEATURE - X=V or A
  SITE 15: note = MISC_FEATURE - X=E or T or H or F or G or D
  SITE 17: note = MISC_FEATURE - X=A or F or Y or M or G or L
  SITE 18: note = MISC_FEATURE - X=R or K or Q or D or T or N or G or I or L or S or A
  SITE 19: note = MISC_FEATURE - X=absent or A or P
  SITE 20: note = MISC_FEATURE - X=absent or F or K
  SITE 21: note = MISC_FEATURE - X=N or S or D or G or T
  SITE 22: note = MISC_FEATURE - X=E or S or A or D or Q or G
  SITE 23: note = MISC_FEATURE - X=Y or G or H or D or F
  SITE 26: note = MISC_FEATURE - X=D or N or E or K or G or T
  SITE 27: note = MISC_FEATURE - X=L or V or E
  SITE 30: note = MISC_FEATURE - X=K or E or D
  SITE 31: note = MISC_FEATURE - X=N or D
  SITE 34: note = MISC_FEATURE - X=K or T or S or E
  SITE 35: note = MISC_FEATURE - X=S or I
  SITE 39: note = MISC_FEATURE - X=Q or N or E
  SITE 40: note = MISC_FEATURE - X=W or I
  SITE 41: note = MISC_FEATURE - X=V or S or L or A or G or Q or F or I
  SITE 43: note = MISC_FEATURE - X=K or R or T or I or P or Q
  SITE 44: note = MISC_FEATURE - X=Y or W or H
  SITE 46: note = MISC_FEATURE - X=N or D
  SITE 47: note = MISC_FEATURE - X=G or A
  SITE 49: note = MISC_FEATURE - X=W or Y or X
  SITE 51: note = MISC_FEATURE - X=K or I or E or Y
  SITE 52: note = MISC_FEATURE - X=E or D or A or K or Q
  SITE 55: note = MISC_FEATURE - X=D or N
  SITE 56: note = MISC_FEATURE - X=N or D or K or S or R or E
  SITE 60: note = MISC_FEATURE - X=R or K
  SITE 61: note = MISC_FEATURE - X=V or I
  SITE 62: note = MISC_FEATURE - X=P or E or W
  SITE 64: note = MISC_FEATURE - X=K or N or R
  SITE 66: note = MISC_FEATURE - X=H or R or Q
XXDXYIAXXXNCXYXCXXXXXXXCNXXCTXXGAXXGYCXXXGXXGXXCXCXXLPXXVPIXXXGXCX

SEQ ID NO: 65 - protein, 64 aa, alpha-like toxin BmK-M1
VRDAYIAKPHNCVYECARNEYCNDLCTKNGAKSGYCQWVGKYGNGCWCIELPDNVPIRVPGKCH

SEQ ID NO: 66 - protein, 36 aa, synthetic construct
  REGION 1..36: note = Consensus sequence for beta/kappa-theraphotoxin-Cg1a
  SITE 1: note = MISC_FEATURE - X=D or E or G or A
  SITE 2: note = MISC_FEATURE - X=G or R
  SITE 3: note = MISC_FEATURE - X=E or Q or A
  SITE 5: note = MISC_FEATURE - X=G or Q
  SITE 6: note = MISC_FEATURE - X=G or E or K
  SITE 7: note = MISC_FEATURE - X=F or Y
  SITE 8: note = MISC_FEATURE - X=W or M
  SITE 9: note = MISC_FEATURE - X=W or R
  SITE 12: note = MISC_FEATURE - X=G or K
  SITE 13: note = MISC_FEATURE - X=R or S or A or N
  SITE 14: note = MISC_FEATURE - X=G or D or S
  SITE 15: note = MISC_FEATURE - X=absent or K
  SITE 16: note = MISC_FEATURE - X=P or N
  SITE 17: note = MISC_FEATURE - X=P or A or T or D
  SITE 20: note = MISC_FEATURE - X=K or P or S
  SITE 21: note = MISC_FEATURE - X=G or K or D
  SITE 22: note = MISC_FEATURE - X=Y or L
  SITE 23: note = MISC_FEATURE - X=A or V or D or E
  SITE 26: note = MISC_FEATURE - X=K or P or S
  SITE 27: note = MISC_FEATURE - X=T or K or R
  SITE 29: note = MISC_FEATURE - X=G or K or R
  SITE 30: note = MISC_FEATURE - X=W or L
  SITE 32: note = MISC_FEATURE - X=A or N or V
  SITE 33: note = MISC_FEATURE - X=V or F or L or W
  SITE 34: note = MISC_FEATURE - X=E or P or K or N or A
  SITE 35: note = MISC_FEATURE - X=A or M or S or P
  SITE 36: note = MISC_FEATURE - X=P or W
XXXCXXXXXKCXXXXXXCCXXXXCSXXWXXCXXXXX

SEQ ID NO: 67 - protein, 36 aa, beta/kappa-theraphotoxin-Cg1a
DGECGGFWWKCGRGKPPCCKGYACSKTWGWCAVEAP

SEQ ID NO: 68 - protein, 34 aa, synthetic construct
  REGION 1..34: note = Consensus sequence for kappa-theraphotoxin-Cg1a
  SITE 3: note = MISC_FEATURE - X=R or K
  SITE 10: note = MISC_FEATURE - X=S or T
  SITE 12: note = MISC_FEATURE - X=D or H
  SITE 32: note = MISC_FEATURE - X=G or L
ECXKMFGGCXVXSDCCAHLGCKPTLKYCAWDXTF

SEQ ID NO: 69 - protein, 34 aa, kappa-theraphotoxin-Cg1a
ECRKMFGGCSVDSDCCAHLGCKPTLKYCAWDGTF

SEQ ID NO: 70 - protein, 64 aa, synthetic construct
  REGION 1..64: note = Consensus sequence for delta-theraphotoxin-Cg1a 1, 2 and 3
  SITE 11: note = MISC_FEATURE - X=S or G
  SITE 15: note = MISC_FEATURE - X=L or V
  SITE 20: note = MISC_FEATURE - X=A or P or V
  SITE 22: note = MISC_FEATURE - X=T or I
  SITE 24: note = MISC_FEATURE - X=I or M
  SITE 26: note = MISC_FEATURE - X=absent or E
  SITE 27: note = MISC_FEATURE - X=absent or E
  SITE 32: note = MISC_FEATURE - X=A or E or G
  SITE 35: note = MISC_FEATURE - X=Q or Y or T
  SITE 36: note = MISC_FEATURE - X=F or M
  SITE 38: note = MISC_FEATURE - X=W or S
  SITE 39: note = MISC_FEATURE - X=K or P
  SITE 41: note = MISC_FEATURE - X=G or S
  SITE 42: note = MISC_FEATURE - X=E or T
  SITE 43: note = MISC_FEATURE - X=G or E
  SITE 44: note = MISC_FEATURE - X=absent or K
  SITE 45: note = MISC_FEATURE - X=P or K
  SITE 49: note = MISC_FEATURE - X=A or T or D
  SITE 50: note = MISC_FEATURE - X=N or G
  SITE 51: note = MISC_FEATURE - X=F or Y
  SITE 52: note = MISC_FEATURE - X=A or S
  SITE 54: note = MISC_FEATURE - X=K or Q
  SITE 55: note = MISC_FEATURE - X=I or P
  SITE 56: note = MISC_FEATURE - X=G or A
  SITE 57: note = MISC_FEATURE - X=L or I
  SITE 58: note = MISC_FEATURE - X=Y or K
  SITE 59: note = MISC_FEATURE - X=L or W
MKTSILFVIFXLALXFALSXAXEXEXXETDRXCGXXWXXCXXXXXPCCXXXXCXXXXXXCIWSP

SEQ ID NO: 71 - protein, 62 aa, delta-theraphotoxin-Cg1a 1
MKTSILFVIFSLALLFALSAATEIEETDRACGQFWWKCGEGKPPCCANFACKIGLYLCIWSP

SEQ ID NO: 72 - protein, 62 aa, delta-theraphotoxin-Cg1a 2; identical to SEQ ID NO: 71

SEQ ID NO: 73 - protein, 62 aa, delta-theraphotoxin-Cg1a 3
MKTSILFVIFSLALVFALSPATEIEETDRACGQFWWKCGEGKPPCCANFACKIGLYLCIWSP

SEQ ID NO: 74 - protein, 66 aa, Muscarinic toxin 1
LTCVTSKSIFGITTENCPDGQNLCFKKWYYIVPRYSDITWGCAATCPKPTNVRETIRCCETDKCNE

SEQ ID NO: 75 - protein, 65 aa, Muscarinic toxin 2
LTCVTTKSIGGVTTEDCPAGQNVCFKRWHYVTPKNYDIIKGCAATCPKVDNNDPIRCCGTDKCND

SEQ ID NO: 76 - protein, 65 aa, Muscarinic toxin 3
LTCVTKNTIFGITTENCPAGQNLCFKRWHYVIPRYTEITRGCAATCPIPENYDSIHCCKTDKCNE

SEQ ID NO: 77 - protein, 65 aa, Muscarinic toxin 7
LTCVKSNSIWFPTSEDCPDGQNLCFKRWQYISPRMYDFTRGCAATCPKAEYRDVINCCGTDKCNK

SEQ ID NO: 78 - protein, 65 aa, Adrenergic toxin rho-elapitoxin-Dp1a
LTCVTSKSIFGITTEDCPDGQNLCFKRRHYVVPKIYDITRGCVATCPIPENYDSIHCCKTDKCNE

SEQ ID NO: 79 - protein, 65 aa, Toxin AdTx1
LTCVTSKSIFGITTEDCPDGQNLCFKRRHYVVPKIYDSTRGCAATCPIPENYDSIHCCKTDKCNE

SEQ ID NO: 80 - protein, 63 aa, synthetic construct
  REGION 1..63: note = Consensus sequence for beta-cardiotoxin
  SITE 13: note = MISC_FEATURE - X=T or K
  SITE 21: note = MISC_FEATURE - X=K or R
  SITE 23: note = MISC_FEATURE - X=V or I
  SITE 41: note = MISC_FEATURE - X=I or T
  SITE 52: note = MISC_FEATURE - X=E or V
  SITE 54: note = MISC_FEATURE - X=L or V
  SITE 62: note = MISC_FEATURE - X=N or D
RKCLNTPLPLIYXTCPIGQDXCXKMTIKKLPSKYDVIRGCXDICPKSSADVXVXCCDTNKCXK

SEQ ID NO: 81 - protein, 63 aa, beta-cardiotoxin
RKCLNTPLPLIYTTCPIGQDKCVKMTIKKLPSKYDVIRGCIDICPKSSADVEVLCCDTNKCNK

SEQ ID NO: 82 - protein, 76 aa, omega-agatoxin-IIIA
SCIDIGGDCDGEKDDCQCCRRNGYCSCYSLFGYLKSGCKCVVGTSAEFQGICRRKARQCYNSDPDKCESHNKPKRR

SEQ ID NO: 83 - protein, 60 aa, calcicludine
WQPPWYCKEPVRIGSCKKQFSSFYFKWTAKKCLPFLFSGCGGNANRFQTIGECRKKCLGK

SEQ ID NO: 84 - protein, 74 aa, omega-filistatoxin-Kh1a
AECLMIGDTSCVPRLGRRCCYGAWCYCDQQLSCRRVGRKRECGWVEVNCKCGWSWSQRIDDWRADYSCKCPEDQ

SEQ ID NO: 85 - protein, 29 aa, beta-theraphotoxin-Gr1a
YCQKWMWTCDSKRKCCEDMVCQLWCKKRL

SEQ ID NO: 86 - protein, 29 aa, beta-theraphotoxin-Gr1b
YCQKWLWTCDSERKCCEDMVCRLWCKKRL

SEQ ID NO: 87 - protein, 31 aa, kappa-theraphotoxin-Gr2c
YCQKWMWTCDEERKCCEGLVCRLWCKKKIEW

SEQ ID NO: 88 - protein, 82 aa, M-theraphotoxin-Gr1a
MKTSVVFVIAGLALLSVVCYASELKEQSSVNEVLSTIFHFEQPEERGCLEFWWKCNPNDDKCCRPKLKCSKLFKLCNFSFGK

SEQ ID NO: 89 - protein, 28 aa, Taicatoxin, alpha-neurotoxin-like component
  SITE 26: note = misc_feature - Xaa can be any naturally occurring amino acid
RRCFITPNVRSERCPPGQEVCFTKTXDG

SEQ ID NO: 90 - protein, 35 aa, beta/omega-theraphotoxin-Tp1a
ECRYWLGGCSAGQTCCKHLVCSRRHGWCVWDGTFS

SEQ ID NO: 91 - protein, 30 aa, beta/omega-theraphotoxin-Tp2a
YCQKWMWTCDSERKCCEGMVCRLWCKKKLW

SEQ ID NO: 92 - protein, 29 aa, beta/kappa-theraphotoxin-Cg2a
YCQKWMWTCDSKRACCEGLRCKLWCRKII

SEQ ID NO: 93 - protein, 35 aa, Mu-theraphotoxin-Hhn1b (1-2-3)
ECLGFGKGCNPSNDQCCKSSNLVCSRKHRWCKYEI

SEQ ID NO: 94 - protein, 35 aa, Mu-theraphotoxin-Hhn1a
ECLGFGKGCNPSNDQCCKSANLVCSRKHRWCKYEI

SEQ ID NO: 95 - protein, 21 aa, mu-conotoxin CnIIIc
ZCCDGPKGCSSKWCRDHARCC